European Patent Specification EP 3 143 538 B1, published January 15, 2025. Title: MODEL ADJUSTMENT DURING ANALYSIS OF A POLYMER FROM NANOPORE MEASUREMENTS. Applicant: OXFORD NANOPORE TECHNOLOGIES LIMITED. The sequence listing filed with the application follows.

SEQUENCE LISTING (16 sequences)

SEQ ID NO: 1 - DNA, 558 bp, Artificial Sequence
  MS-(B1)8 = MS-(D90N/D91N/D93N/D118R/D134R/E139K)8
atgggtctggataatgaactgagcctggtggacggtcaagatcgtaccctgacggtgcaacaatgggatacctttctgaatggcgtttttccgctggatcgtaatcgcctgacccgtgaatggtttcattccggtcgcgcaaaatatatcgtcgcaggcccgggtgctgacgaattcgaaggcacgctggaactgggttatcagattggctttccgtggtcactgggcgttggtatcaacttctcgtacaccacgccgaatattctgatcaacaatggtaacattaccgcaccgccgtttggcctgaacagcgtgattacgccgaacctgtttccgggtgttagcatctctgcccgtctgggcaatggtccgggcattcaagaagtggcaacctttagtgtgcgcgtttccggcgctaaaggcggtgtcgcggtgtctaacgcccacggtaccgttacgggcgcggccggcggtgtcctgctgcgtccgttcgcgcgcctgattgcctctaccggcgacagcgttacgacctatggcgaaccgtggaatatgaactaa

SEQ ID NO: 2 - protein, 184 aa, Artificial Sequence
  MS-(B1)8 = MS-(D90N/D91N/D93N/D118R/D134R/E139K)8
GLDNELSLVDGQDRTLTVQQWDTFLNGVFPLDRNRLTREWFHSGRAKYIVAGPGADEFEGTLELGYQIGFPWSLGVGINFSYTTPNILINNGNITAPPFGLNSVITPNLFPGVSISARLGNGPGIQEVATFSVRVSGAKGGVAVSNAHGTVTGAAGGVLLRPFARLIASTGDSVTTYGEPWNMN

SEQ ID NO: 3 - DNA, 558 bp, Artificial Sequence
  MS-(B2)8 = MS-(L88N/D90N/D91N/D93N/D118R/D134R/E139K)8
atgggtctggataatgaactgagcctggtggacggtcaagatcgtaccctgacggtgcaacaatgggatacctttctgaatggcgtttttccgctggatcgtaatcgcctgacccgtgaatggtttcattccggtcgcgcaaaatatatcgtcgcaggcccgggtgctgacgaattcgaaggcacgctggaactgggttatcagattggctttccgtggtcactgggcgttggtatcaacttctcgtacaccacgccgaatattaacatcaacaatggtaacattaccgcaccgccgtttggcctgaacagcgtgattacgccgaacctgtttccgggtgttagcatctctgcccgtctgggcaatggtccgggcattcaagaagtggcaacctttagtgtgcgcgtttccggcgctaaaggcggtgtcgcggtgtctaacgcccacggtaccgttacgggcgcggccggcggtgtcctgctgcgtccgttcgcgcgcctgattgcctctaccggcgacagcgttacgacctatggcgaaccgtggaatatgaactaa

SEQ ID NO: 4 - protein, 184 aa, Artificial Sequence
  MS-(B2)8 = MS-(L88N/D90N/D91N/D93N/D118R/D134R/E139K)8
GLDNELSLVDGQDRTLTVQQWDTFLNGVFPLDRNRLTREWFHSGRAKYIVAGPGADEFEGTLELGYQIGFPWSLGVGINFSYTTPNININNGNITAPPFGLNSVITPNLFPGVSISARLGNGPGIQEVATFSVRVSGAKGGVAVSNAHGTVTGAAGGVLLRPFARLIASTGDSVTTYGEPWNMN

SEQ ID NO: 5 - protein, 485 aa, Escherichia coli
MMNDGKQQSTFLFHDYETFGTHPALDRPAQFAAIRTDSEFNVIGEPEVFYCKPADDYLPQPGAVLITGITPQEARAKGENEAAFAARIHSLFTVPKTCILGYNNVRFDDEVTRNIFYRNFYDPYAWSWQHDNSRWDLLDVMRACYALRPEGINWPENDDGLPSFRLEHLTKANGIEHSNAHDAMADVYATIAMAKLVKTRQPRLFDYLFTHRNKHKLMALIDVPQMKPLVHVSGMFGAWRGNTSWVAPLAWHPENRNAVIMVDLAGDISPLLELDSDTLRERLYTAKTDLGDNAAVPVKLVHINKCPVLAQANTLRPEDADRLGINRQHCLDNLKILRENPQVREKVVAIFAEAEPFTPSDNVDAQLYNGFFSDADRAAMKIVLETEPRNLPALDITFVDKRIEKLLFNYRARNFPGTLDYAEQQRWLEHRRQVFTPEFLQGYADELQMLVQQYADDKEKVALLKALWQYAEEIVSGSGHHHHHH

SEQ ID NO: 6 - protein, 268 aa, Escherichia coli
MKFVSFNINGLRARPHQLEAIVEKHQPDVIGLQETKVHDDMFPLEEVAKLGYNVFYHGQKGHYGVALLTKETPIAVRRGFPGDDEEAQRRIIMAEIPSLLGNVTVINGYFPQGESRDHPIKFPAKAQFYQNLQNYLETELKRDNPVLIMGDMNISPTDLDIGIGEENRKRWLRTGKCSFLPEEREWMDRLMSWGLVDTFRHANPQTADRFSWFDYRSKGFDDNRGLRIDLLLASQPLAECCVETGIDYEIRSMEKPSDHAPVWATFRR

SEQ ID NO: 7 - protein, 666 aa, Thermus thermophilus
MRDRVRWRVLSLPPLAQWREVMAALEVGPEAALAYWHRGFRRKEDLDPPLALLPLKGLREAAALLEEALRQGKRIRVHGDYDADGLTGTAILVRGLAALGADVHPFIPHRLEEGYGVLMERVPEHLEASDLFLTVDCGITNHAELRELLENGVEVIVTDHHTPGKTPSPGLVVHPALTPDLKEKPTGAGVVFLLLWALHERLGLPPPLEYADLAAVGTIADVAPLWGWNRALVKEGLARIPASSWVGLRLLAEAVGYTGKAVEVAFRIAPRINAASRLGEAEKALRLLLTDDAAEAQALVGELHRLNARRQTLEEAMLRKLLPQADPEAKAIVLLDPEGHPGVMGIVASRILEATLRPVFLVAQGKGTVRSLAPISAVEALRSAEDLLLRYGGHKEAAGFAMDEALFPAFKARVEAYAARFPDPVREVALLDLLPEPGLLPQVFRELALLEPYGEGNPEPLFLLFGAPEEARRLGEGRHLAFRLKGVRVLAWKQGDLALPPEVEVAGLLSENAWNGHLAYEVQAVDLRKPEALEGGIAPFAYPLPLLEALARARLGEGVYVPEDNPEGLDYARKAGFRLLPPEEAGLWLGLPPRPVLGRRVEVALGREARARLSAPPVLHTPEARLKALVHRRLLFAYERRHPGLFSEALLAYWEVNRVQEPAGSP

SEQ ID NO: 8 - protein, 226 aa, Bacteriophage lambda
MTPDIILQRTGIDVRAVEQGDDAWHKLRLGVITASEVHNVIAKPRSGKKWPDMKMSYFHTLLAEVCTGVAPEVNAKALAWGKQYENDARTLFEFTSGVNVTESPIIYRDESMRTACSPDGLCSDGNGLELKCPFTSRDFMKFRLGGFEAIKSAYMAQVQYSMWVTRKNAWYFANYDPRMKREGLHYVVIERDEKYMASFDEIVPEFIEKMDEALAEIGFVFGEQWR

SEQ ID NO: 9 - protein, 608 aa, Bacteriophage phi-29
MKHMPRKMYSCAFETTTKVEDCRVWAYGYMNIEDHSEYKIGNSLDEFMAWVLKVQADLYFHNLKFDGAFIINWLERNGFKWSADGLPNTYNTIISRMGQWYMIDICLGYKGKRKIHTVIYDSLKKLPFPVKKIAKDFKLTVLKGDIDYHKERPVGYKITPEEYAYIKNDIQIIAEALLIQFKQGLDRMTAGSDSLKGFKDIITTKKFKKVFPTLSLGLDKEVRYAYRGGFTWLNDRFKEKEIGEGMVFDVNSLYPAQMYSRLLPYGEPIVFEGKYVWDEDYPLHIQHIRCEFELKEGYIPTIQIKRSRFYKGNEYLKSSGGEIADLWLSNVDLELMKEHYDLYNVEYISGLKFKATTGLFKDFIDKWTYIKTTSEGAIKQLAKLMLNSLYGKFASNPDVTGKVPYLKENGALGFRLGEEETKDPVYTPMGVFITAWARYTTITAAQACYDRIIYCDTDSIHLTGTEIPDVIKDIVDPKKLGYWAHESTFKRAKYLRQKTYIQDIYMKEVDGKLVEGSPDDYTDIKFSVKCAGMTDKIKKEVTFENFKVGFSRKMKPKPVQVPGGVVLVDDTFTIKSGGSAWSHPQFEKGGGSGGGSGGSAWSHPQFEK

SEQ ID NO: 10 - protein, 760 aa, Methanococcoides burtonii
MMIRELDIPRDIIGFYEDSGIKELYPPQAEAIEMGLLEKKNLLAAIPTASGKTLLAELAMIKAIREGGKALYIVPLRALASEKFERFKELAPFGIKVGISTGDLDSRADWLGVNDIIVATSEKTDSLLRNGTSWMDEITTVVVDEIHLLDSKNRGPTLEVTITKLMRLNPDVQVVALSATVGNAREMADWLGAALVLSEWRPTDLHEGVLFGDAINFPGSQKKIDRLEKDDAVNLVLDTIKAEGQCLVFESSRRNCAGFAKTASSKVAKILDNDIMIKLAGIAEEVESTGETDTAIVLANCIRKGVAFHHAGLNSNHRKLVENGFRQNLIKVISSTPTLAAGLNLPARRVIIRSYRRFDSNFGMQPIPVLEYKQMAGRAGRPHLDPYGESVLLAKTYDEFAQLMENYVEADAEDIWSKLGTENALRTHVLSTIVNGFASTRQELFDFFGATFFAYQQDKWMLEEVINDCLEFLIDKAMVSETEDIEDASKLFLRGTRLGSLVSMLYIDPLSGSKIVDGFKDIGKSTGGNMGSLEDDKGDDITVTDMTLLHLVCSTPDMRQLYLRNTDYTIVNEYIVAHSDEFHEIPDKLKETDYEWFMGEVKTAMLLEEWVTEVSAEDITRHFNVGEGDIHALADTSEWLMHAAAKLAELLGVEYSSHAYSLEKRIRYGSGLDLMELVGIRGVGRVRARKLYNAGFVSVAKLKGADISVLSKLVGPKVAYNILSGIGVRVNDKHFNSAPISSNTLDTLLDKNQKTFNDFQ

SEQ ID NO: 11 - protein, 707 aa, Cenarchaeum symbiosum
MRISELDIPRPAIEFLEGEGYKKLYPPQAAAAKAGLTDGKSVLVSAPTASGKTLIAAIAMISHLSRNRGKAVYLSPLRALAAEKFAEFGKIGGIPLGRPVRVGVSTGDFEKAGRSLGNNDILVLTNERMDSLIRRRPDWMDEVGLVIADEIHLIGDRSRGPTLEMVLTKLRGLRSSPQVVALSATISNADEIAGWLDCTLVHSTWRPVPLSEGVYQDGEVAMGDGSRHEVAATGGGPAVDLAAESVAEGGQSLIFADTRARSASLAAKASAVIPEAKGADAAKLAAAAKKIISSGGETKLAKTLAELVEKGAAFHHAGLNQDCRSVVEEEFRSGRIRLLASTPTLAAGVNLPARRVVISSVMRYNSSSGMSEPISILEYKQLCGRAGRPQYDKSGEAIVVGGVNADEIFDRYIGGEPEPIRSAMVDDRALRIHVLSLVTTSPGIKEDDVTEFFLGTLGGQQSGESTVKFSVAVALRFLQEEGMLGRRGGRLAATKMGRLVSRLYMDPMTAVTLRDAVGEASPGRMHTLGFLHLVSECSEFMPRFALRQKDHEVAEMMLEAGRGELLRPVYSYECGRGLLALHRWIGESPEAKLAEDLKFESGDVHRMVESSGWLLRCIWEISKHQERPDLLGELDVLRSRVAYGIKAELVPLVSIKGIGRVRSRRLFRGGIKGPGDLAAVPVERLSRVEGIGATLANNIKSQLRKGG

SEQ ID NO: 12 - protein, 799 aa, Methanospirillum hungatei
MEIASLPLPDSFIRACHAKGIRSLYPPQAECIEKGLLEGKNLLISIPTASGKTLLAEMAMWSRIAAGGKCLYIVPLRALASEKYDEFSKKGVIRVGIATGDLDRTDAYLGENDIIVATSEKTDSLLRNRTPWLSQITCIVLDEVHLIGSENRGATLEMVITKLRYTNPVMQIIGLSATIGNPAQLAEWLDATLITSTWRPVDLRQGVYYNGKIRFSDSERPIQGKTKHDDLNLCLDTIEEGGQCLVFVSSRRNAEGFAKKAAGALKAGSPDSKALAQELRRLRDRDEGNVLADCVERGAAFHHAGLIRQERTIIEEGFRNGYIEVIAATPTLAAGLNLPARRVIIRDYNRFASGLGMVPIPVGEYHQMAGRAGRPHLDPYGEAVLLAKDAPSVERLFETFIDAEAERVDSQCVDDASLCAHILSLIATGFAHDQEALSSFMERTFYFFQHPKTRSLPRLVADAIRFLTTAGMVEERENTLSATRLGSLVSRLYLNPCTARLILDSLKSCKTPTLIGLLHVICVSPDMQRLYLKAADTQLLRTFLFKHKDDLILPLPFEQEEEELWLSGLKTALVLTDWADEFSEGMIEERYGIGAGDLYNIVDSGKWLLHGTERLVSVEMPEMSQVVKTLSVRVHHGVKSELLPLVALRNIGRVRARTLYNAGYPDPEAVARAGLSTIARIIGEGIARQVIDEITGVKRSGIHSSDDDYQQKTPELLTDIPGIGKKMAEKLQNAGIITVSDLLTADEVLLSDVLGAARARKVLAFLSNSEKENSSSDKTEEIPDTQKIRGQSSWEDFGC

SEQ ID NO: 13 - protein, 1756 aa, Escherichia coli
MMSIAQVRSAGSAGNYYTDKDNYYVLGSMGERWAGKGAEQLGLQGSVDKDVFTRLLEGRLPDGADLSRMQDGSNKHRPGYDLTFSAPKSVSMMAMLGGDKRLIDAHNQAVDFAVRQVEALASTRVMTDGQSETVLTGNLVMALFNHDTSRDQEPQLHTHAVVANVTQHNGEWKTLSSDKVGKTGFIENVYANQIAFGRLYREKLKEQVEALGYETEVVGKHGMWEMPGVPVEAFSGRSQAIREAVGEDASLKSRDVAALDTRKSKQHVDPEIRMAEWMQTLKETGFDIRAYRDAADQRTEIRTQAPGPASQDGPDVQQAVTQAIAGLSERKVQFTYTDVLARTVGILPPENGVIERARAGIDEAISREQLIPLDREKGLFTSGIHVLDELSVRALSRDIMKQNRVTVHPEKSVPRTAGYSDAVSVLAQDRPSLAIVSGQGGAAGQRERVAELVMMAREQGREVQIIAADRRSQMNLKQDERLSGELITGRRQLLEGMAFTPGSTVIVDQGEKLSLKETLTLLDGAARHNVQVLITDSGQRTGTGSALMAMKDAGVNTYRWQGGEQRPATIISEPDRNVRYARLAGDFAASVKAGEESVAQVSGVREQAILTQAIRSELKTQGVLGHPEVTMTALSPVWLDSRSRYLRDMYRPGMVMEQWNPETRSHDRYVIDRVTAQSHSLTLRDAQGETQVVRISSLDSSWSLFRPEKMPVADGERLRVTGKIPGLRVSGGDRLQVASVSEDAMTVVVPGRAEPASLPVSDSPFTALKLENGWVETPGHSVSDSATVFASVTQMAMDNATLNGLARSGRDVRLYSSLDETRTAEKLARHPSFTVVSEQIKARAGETLLETAISLQKAGLHTPAQQAIHLALPVLESKNLAFSMVDLLTEAKSFAAEGTGFTELGGEINAQIKRGDLLYVDVAKGYGTGLLVSRASYEAEKSILRHILEGKEAVTPLMERVPGELMETLTSGQRAATRMILETSDRFTVVQGYAGVGKTTQFRAVMSAVNMLPASERPRVVGLGPTHRAVGEMRSAGVDAQTLASFLHDTQLQQRSGETPDFSNTLFLLDESSMVGNTEMARAYALIAAGGGRAVASGDTDQLQAIAPGQSFRLQQTRSAADVVIMKEIVRQTPELREAVYSLINRDVERALSGLESVKPSQVPRLEGAWAPEHSVTEFSHSQEAKLAEAQQKAMLKGEAFPDIPMTLYEAIVRDYTGRTPEAREQTLIVTHLNEDRRVLNSMIHDAREKAGELGKEQVMVPVLNTANIRDGELRRLSTWEKNPDALALVDNVYHRIAGISKDDGLITLQDAEGNTRLISPREAVAEGVTLYTPDKIRVGTGDRMRFTKSDRERGYVANSVWTVTAVSGDSVTLSDGQQTRVIRPGQERAEQHIDLAYAITAHGAQGASETFAIALEGTEGNRKLMAGFESAYVALSRMKQHVQVYTDNRQGWTDAINNAVQKGTAHDVLEPKPDREVMNAQRLFSTARELRDVAAGRAVLRQAGLAGGDSPARFIAPGRKYPQPYVALPAFDRNGKSAGIWLNPLTTDDGNGLRGFSGEGRVKGSGDAQFVALQGSRNGESLLADNMQDGVRIARDNPDSGVVVRIAGEGRPWNPGAITGGRVWGDIPDNSVQPGAGNGEPVTAEVLAQRQAEEAIRRETERRADEIVRKMAENKPDLPDGKTELAVRDIAGQERDRSAISERETALPESVLRESQREREAVREVARENLLQERLQQMERDMVRDLQKEKTLGGD

SEQ ID NO: 14 - protein, 726 aa, Methanococcoides burtonii
MSDKPAFMKYFTQSSCYPNQQEAMDRIHSALMQQQLVLFEGACGTGKTLSALVPALHVGKMLGKTVIIATNVHQQMVQFINEARDIKKVQDVKVAVIKGKTAMCPQEADYEECSVKRENTFELMETEREIYLKRQELNSARDSYKKSHDPAFVTLRDELSKEIDAVEEKARGLRDRACNDLYEVLRSDSEKFREWLYKEVRSPEEINDHAIKDGMCGYELVKRELKHADLLICNYHHVLNPDIFSTVLGWIEKEPQETIVIFDEAHNLESAARSHSSLSLTEHSIEKAITELEANLDLLADDNIHNLFNIFLEVISDTYNSRFKFGERERVRKNWYDIRISDPYERNDIVRGKFLRQAKGDFGEKDDIQILLSEASELGAKLDETYRDQYKKGLSSVMKRSHIRYVADFMSAYIELSHNLNYYPILNVRRDMNDEIYGRVELFTCIPKNVTEPLFNSLFSVILMSATLHPFEMVKKTLGITRDTCEMSYGTSFPEEKRLSIAVSIPPLFAKNRDDRHVTELLEQVLLDSIENSKGNVILFFQSAFEAKRYYSKIEPLVNVPVFLDEVGISSQDVREEFFSIGEENGKAVLLSYLWGTLSEGIDYRDGRGRTVIIIGVGYPALNDRMNAVESAYDHVFGYGAGWEFAIQVPTIRKIRQAMGRVVRSPTDYGARILLDGRFLTDSKKRFGKFSVFEVFPPAERSEFVDVDPEKVKYSLMNFFMDNDEQ

SEQ ID NO: 15 - protein, 439 aa, Dickeya dadantii
MTFDDLTEGQKNAFNIVMKAIKEKKHHVTINGPAGTGKTTLTKFIIEALISTGETGIILAAPTHAAKKILSKLSGKEASTIHSILKINPVTYEENVLFEQKEVPDLAKCRVLICDEVSMYDRKLFKILLSTIPPWCTIIGIGDNKQIRPVDPGENTAYISPFFTHKDFYQCELTEVKRSNAPIIDVATDVRNGKWIYDKVVDGHGVRGFTGDTALRDFMVNYFSIVKSLDDLFENRVMAFTNKSVDKLNSIIRKKIFETDKDFIVGEIIVMQEPLFKTYKIDGKPVSEIIFNNGQLVRIIEAEYTSTFVKARGVPGEYLIRHWDLTVETYGDDEYYREKIKIISSDEELYKFNLFLGKTAETYKNWNKGGKAPWSDFWDAKSQFSKVKALPASTFHKAQGMSVDRAFIYTPCIHYADVELAQQLLYVGVTRGRYDVFYV

SEQ ID NO: 16 - protein, 970 aa, Clostridium botulinum
MLSVANVRSPSAAASYFASDNYYASADADRSGQWIGDGAKRLGLEGKVEARAFDALLRGELPDGSSVGNPGQAHRPGTDLTFSVPKSWSLLALVGKDERIIAAYREAVVEALHWAEKNAAETRVVEKGMVVTQATGNLAIGLFQHDTNRNQEPNLHFHAVIANVTQGKDGKWRTLKNDRLWQLNTTLNSIAMARFRVAVEKLGYEPGPVLKHGNFEARGISREQVMAFSTRRKEVLEARRGPGLDAGRIAALDTRASKEGIEDRATLSKQWSEAAQSIGLDLKPLVDRARTKALGQGMEATRIGSLVERGRAWLSRFAAHVRGDPADPLVPPSVLKQDRQTIAAAQAVASAVRHLSQREAAFERTALYKAALDFGLPTTIADVEKRTRALVRSGDLIAGKGEHKGWLASRDAVVTEQRILSEVAAGKGDSSPAITPQKAAASVQAAALTGQGFRLNEGQLAAARLILISKDRTIAVQGIAGAGKSSVLKPVAEVLRDEGHPVIGLAIQNTLVQMLERDTGIGSQTLARFLGGWNKLLDDPGNVALRAEAQASLKDHVLVLDEASMVSNEDKEKLVRLANLAGVHRLVLIGDRKQLGAVDAGKPFALLQRAGIARAEMATNLRARDPVVREAQAAAQAGDVRKALRHLKSHTVEARGDGAQVAAETWLALDKETRARTSIYASGRAIRSAVNAAVQQGLLASREIGPAKMKLEVLDRVNTTREELRHLPAYRAGRVLEVSRKQQALGLFIGEYRVIGQDRKGKLVEVEDKRGKRFRFDPARIRAGKGDDNLTLLEPRKLEIHEGDRIRWTRNDHRRGLFNADQARVVEIANGKVTFETSKGDLVELKKDDPMLKRIDLAYALNVHMAQGLTSDRGIAVMDSRERNLSNQKTFLVTVTRLRDHLTLVVDSADKLGAAVARNKGEKASAIEVTGSVKPTATKGSGVDQPKSVEANKAEKELTRSKSKTLDFGI